European Patent Specification EP 3 894 599 B1, published March 19, 2025. Title: pks-island positive E.coli as marker of negative response to anti-PD1 therapy in colorectal cancer. Applicant: SANOFI Université Clermont Auvergne. The sequence listing filed with the application follows.

SEQUENCE LISTING (4 sequences)

SEQ ID NO: 1 - DNA, 24 bp, Artificial Sequence
  ClbN forward primer
gttttgctcgccagatagtcattc

SEQ ID NO: 2 - DNA, 22 bp, Artificial Sequence
  ClbN reverse primer
cagttcgggtatgtgtggaagg

SEQ ID NO: 3 - protein, 218 aa, Artificial Sequence
  RPM1-14 light chain, without SP chimeric mouse Variable  rat Constant Kappa
DIVMTQGTLPNPVPSGESVSITCRSSKSLLYSDGKTYLNWYLQRPGQSPQLLIYWMSTRASGVSDRFSGSGSGTDFTLKISGVEAEDVGIYYCQQGLEFPTFGGGTKLELKRADAAPTVSIFPPSSEQLTSGGASVVCFLNNFYPKDINVKWKIDGSERQNGVLNSWTDQDSKDSTYSMSSTLTLTKDEYERHNSYTCEATHKTSTSPIVKSFNRNEC

SEQ ID NO: 4 - protein, 443 aa, Artificial Sequence
  RMP1-14 heavy chain, without  SP mouse variable, mouse constant IgG1
EVQLQESGPGLVKPSQSLSLTCSVTGYSITSSYRWNWIRKFPGNRLEWMGYINSAGISNYNPSLKRRISITRDTSKNQFFLQVNSVTTEDAATYYCARSDNMGTTPFTYWGQGTLVTVSSAKTTPPSVYPLAPGSAAQTNSMVTLGCLVKGYFPEPVTVTWNSGSLSSGVHTFPAVLQSDLYTLSSSVTVPSSTWPSETVTCNVAHPASSTKVDKKIVPRDCGCKPCICTVPEVSSVFIFPPKPKDVLTITLTPKVTCVVVDISKDDPEVQFSWFVDDVEVHTAQTQPREEQFNSTFRSVSELPIMHQDWLNGKEFKCRVNSAAFPAPIEKTISKTKGRPKAPQVYTIPPPKEQMAKDKVSLTCMITDFFPEDITVEWQWNGQPAENYKNTQPIMDTDGSYFVYSKLNVQKSNWEAGNTFTCSVLHEGLHNHHTEKSLSHSPG